European Patent Specification EP 3 384 934 B1, published August 23, 2023. Title: Endocytosis enhancer by using agglutinate molecule. Applicant: Quarrymen & Co. Inc Saitama University. The sequence listing filed with the application follows.

SEQUENCE LISTING (34 sequences)

SEQ ID NO: 1 - protein, 10 aa, Homo sapiens
  PEPTIDE (1)..(10): MCF7-1
DMPGTVLPGG

SEQ ID NO: 2 - protein, 10 aa, Homo sapiens
  PEPTIDE (1)..(10): MCF7-2
VPTDTDYSGG

SEQ ID NO: 3 - protein, 29 aa, Homo sapiens
  PEPTIDE (1)..(29): MCF7-1+alpha stand peptide
DMPGTVLPGGGGGSEGEWQQQQHQWAKQE

SEQ ID NO: 4 - protein, 272 aa, Aequorea victoria
  PEPTIDE (1)..(272)
MASMTGGQQMGRDMPGTVLPGGMSKGEELFTGVVPILVELDGDVNGHKFSVSGEGEGDATYGKLTLKFISTTGKLPVPWPTLVTTLTYGVQCFSRYPDHMKRHDFFKSAMPEGYVQERTISFKDDGNYKTRAEVKFEGDTLVNRIELKGIDFKEDGNILGHKLEYNYNSHNVYITADKQRNGIKANFKTRHNIEDGSVQLADHYQQNTPIGDGPVLLPDNHYLSTQSALLKDPNEKRDHMVLLEFVTAAGSGITDEVDGTELYKGGHHHHHH

SEQ ID NO: 5 - protein, 272 aa, Aequorea victoria
  PEPTIDE (1)..(272)
MASMTGGQQMGRVPTDTDYSGGMSKGEELFTGVVPILVELDGDVNGHKFSVSGEGEGDATYGKLTLKFISTTGKLPVPWPTLVTTLTYGVQCFSRYPDHMKRHDFFKSAMPEGYVQERTISFNDDGNYKTRAEVKFEGDTLVNRIELKGIDFKEDGNILGHKLEYNYNSHNVYITADKQRNGIKANFKTRHNIEDGSVQLADHYQQNTPIGDGPVLLPDNHYLSTQSALLKDPNDKRDHMVLLEFVTAAGSGITDEVDGTELYKGGHHHHHH

SEQ ID NO: 6 - protein, 292 aa, Aequorea victoria
  PEPTIDE (1)..(292)
MASMTGGQQMGRDMPGTVLPGGGGGSEGEWQQQQHQWAKQEMSKGEELFTGVVPILVELDGDVNGHKFSVSGEGEGDATYGKLTLKFISTTGKLPVPWPTLVTTLTYGVQCFSRYPDHMKRHDFFKSAMPEGYVQERTISFKDDGNYKTRAEVKFEGDTLVNRIELKGIDFKEDGNILGHKLEYNYNSHNVYITADKQRNGIKANFKTRHNIEDGSVQLADHYQQNTPIGDGPVLLPDNHYLSTQSALLKDPNEKRDHMVLLEFVTAAGSGITDEVDGTCELYKGGHHHHHH

SEQ ID NO: 7 - protein, 263 aa, Aequorea victoria
  PEPTIDE (1)..(263): GFP
MASMTGGQQMGRMSKGEELFTGVVPILVELDGDVNGHKFSVSGEGEGDATYGKLTLKFISTTGKLPVPWPTLVTTLTYGVQCFSRYPDHMKRHDFFKSAMPEGYVQERTISFKDDGNYKTRAEVKFEGDTLVNRIELKGIDFKEDGNILGHKLEYNYNSHNVYITADKQKNGIKANFKTRHNIEDGSVQLADHYQQNTPIGDGPVLLPDNHYLSTQSALLKDPNEKRDHMVLLEFVTAAGSGITDEVDGTCELYKGGHHHHHH

SEQ ID NO: 8 - protein, 258 aa, Aequorea victoria
  PEPTIDE (1)..(258): GFP
MASMTGGQQMGRMSKGEELFTGVVPILVELDGDVNGHKFSVSGEGEGDATYGKLTLKFICTTGKLPVPWPTLVTTLTYGVQCFSRYPDHMKRHDFFKSAMPEGYVQERTISFKDDGNYKTRAEVKFEGDTLVNRIELKGIDFKEDGNILGHKLEYNYNSHNVYITADKQKNGIKANFKTRHNIEDGSVQLADHYQQNTPIGDGPVLLPDNHYLSTQSALLKDPNEKRDHMVLLEFVTAAGITHGMDELYKGGHHHHHH

SEQ ID NO: 9 - protein, 259 aa, Aequorea victoria
  PEPTIDE (1)..(259): GFP
MASMTGGQQMGRMVSKGEELFTGVVPILVELDGDVNGHKFSVSGEGEGDATYGKLTLKFICTTGKLPVPWPTLVTTLTHGVQCFSRYPDHMKQHDFFKSAMPEGYVQERTIFFKDDGNYKTRAEVKFEGDTLVNRIELKGIDFKEDGNILGHKLEYNFNSHNVYIMADKQKNGIKVNFKIRHNIEDGSVQLADHYQQNTPIGDGPVLLPDNHYLSTQSALSKDPNEKRDHMVLLEFVTAAGITLGMDELYKGGHHHHHH

SEQ ID NO: 10 - protein, 259 aa, Aequorea victoria
  PEPTIDE (1)..(259)
MASMTGGQQMGRMVSKGEELFTGVVPILVELDGDVNGHKFSVSGEGEGDATYGKLTLKFICTTGKLPVPWPTLVTTFGYGLQCFARYPDHMKQHDFFKSAMPEGYVQERTIFFKDDGNYKTRAEVKFEGDTLVNRIELKGIDFKEDGNILGHKLEYNYNSHNVYIMADKQKNGIKVNFKIRHNIEDGSVQLADHYQQNTPIGDGPVLLPDNHYLSYQSALSKDPNEKRDHMVLLEFVTAAGITLGMDELYKGGHHHHHH

SEQ ID NO: 11 - protein, 236 aa, Actinia equina
  PEPTIDE (1)..(236)
  PEPTIDE (1)..(236): GFP
MASSEDVIKEFMRFKVRMEGSVNGHEFEIEGEGEGRPYEGTQTAKLKVTKGGPLPFAWDILSPQFQYGSKVYVKHPADIPDYKKLSFPEGFKWERVMNFEDGGVVTVTQDSSLQDGCFIYKVKFIGVNFPSDGPVMQKKTMGWEPSTERLYPRDGVLKGEIHKALKLKDGGHYLVEFKSIYMAKKPVQLPGYYYVDSKLDITSHNEDYTIVEQYERTEGRHHLFLGTCGGHHHHHH

SEQ ID NO: 12 - DNA, 45 bp, Artificial Sequence
  Primer
  prim_transcript (1)..(45)
cctggtactgttcttcctggtggtatgagtaaaggagaagaactt

SEQ ID NO: 13 - DNA, 27 bp, Artificial Sequence
  primer
  prim_transcript (1)..(27): Primer
catatcgcgacccatttgctgtccacc

SEQ ID NO: 14 - DNA, 45 bp, Artificial Sequence
  Primer
  prim_transcript (1)..(45): Primer for MCF7-1
actgatactgattatagtggaggaatgagtaaaggagaagaactt

SEQ ID NO: 15 - DNA, 27 bp, Artificial Sequence
  Primer
  prim_transcript (1)..(27): Primer for MCF7-1
aggaacgcgacccatttgctgtccacc

SEQ ID NO: 16 - DNA, 51 bp, Artificial Sequence
  Primer
  prim_transcript (1)..(51): Primer for MCF7-2
caacaacaacaacatcaatgggcaaaacaagaaatgagtaaaggagaagaa

SEQ ID NO: 17 - DNA, 42 bp, Artificial Sequence
  Primer
  prim_transcript (1)..(42): Primer for MCF7-2
ccattcaccttcactaccaccaccaccaccaggaagaacagt

SEQ ID NO: 18 - DNA, 22 bp, Artificial Sequence
  Primer
  prim_transcript (1)..(22): Primer for MCF7-1+alpha stand peptide
cattgaagatggctccgttcaa

SEQ ID NO: 19 - DNA, 22 bp, Artificial Sequence
  Primer
  prim_transcript (1)..(22): Primer for MCF7-1+alpha stand peptide
ttgtggcgagttttgaagttag

SEQ ID NO: 20 - DNA, 70 bp, Artificial Sequence
  Primer for inverse PCR
  prim_transcript (1)..(70): Primer for inverse PCR
ctcgaccatatggctagcatgactggtggacagcaaatgggtcgcatgagtaaaggagaagaacttttca

SEQ ID NO: 21 - DNA, 54 bp, Artificial Sequence
  Primer
  prim_transcript (1)..(54): Primer for inverse PCR
tgacgtgaattcattagtgatggtgatggtgatgtttgtagagctcatccatgc

SEQ ID NO: 22 - DNA, 25 bp, Artificial Sequence
  Primer
  prim_transcript (1)..(25): Primer for inverse PCR
  misc_feature (13)..(14): n is a, c, g, or t
cttaaatttattnnkactggaaaac

SEQ ID NO: 23 - DNA, 20 bp, Artificial Sequence
  Primer
  prim_transcript (1)..(20): Primer for inverse PCR
ggtaagttttccgtatgttg

SEQ ID NO: 24 - DNA, 26 bp, Artificial Sequence
  Oligonucleotide
  misc_binding (1)..(26)
  misc_feature (9)..(10): n is a, c, g, or t
gtgttcaannkttttcccgttatccg

SEQ ID NO: 25 - DNA, 22 bp, Artificial Sequence
  Oligonucleotide
  misc_binding (1)..(22)
catacgtcagagtagtgacaag

SEQ ID NO: 26 - DNA, 23 bp, Artificial Sequence
  Oligonucleotide
  misc_binding (1)..(23)
tgtcttttcactggagttgtccc

SEQ ID NO: 27 - DNA, 21 bp, Artificial Sequence
  Oligonucleotide
  misc_binding (1)..(21)
ttctcctttactcattttttc

SEQ ID NO: 28 - DNA, 24 bp, Artificial Sequence
  Primer
  prim_transcript (1)..(24): Primer for inverse PCR
tgcacacatggcatggatgagctc

SEQ ID NO: 29 - DNA, 21 bp, Artificial Sequence
  Primer
  prim_transcript (1)..(21): Primer for inverse PCR
cccagcagcagttacaaactc

SEQ ID NO: 30 - DNA, 33 bp, Artificial Sequence
  Primer
  prim_transcript (1)..(33): Primer for inverse PCR
cagcgccgttgtgagctctacaaataatgaatt

SEQ ID NO: 31 - DNA, 21 bp, Artificial Sequence
  Primer
  prim_transcript (1)..(21): Primer for inverse PCR
tgtaatcccagcagcagttac

SEQ ID NO: 32 - DNA, 21 bp, Artificial Sequence
  Primer
  prim_transcript (1)..(21): Primer for inverse PCR
acatgtgagctctacaaataa

SEQ ID NO: 33 - DNA, 18 bp, Artificial Sequence
  Primer
  prim_transcript (1)..(18)
acggccctgtgtaatccc

SEQ ID NO: 34 - DNA, 21 bp, Artificial Sequence
  Primer
  prim_transcript (1)..(21): Primer for inverse PCR
ggaacatgtgagctctacaaa